European Patent Specification EP 3 485 022 B1, published April 2, 2025. Title: Plants comprising wheat G-type cytoplasmic male sterility restorer genes, molecular markers and uses thereof. Applicant: Bayer CropScience NV. The sequence listing filed with the application follows.

SEQUENCE LISTING (26 sequences)

SEQ ID NO: 1 - DNA, 101 bp, Triticum aestivum
acctttatcgtctcttggtactgtgatattgagactggtaagtaaggttcrgttggtgcttaatcaccataggccatagcatgggccctgtcctagtgtaa

SEQ ID NO: 2 - DNA, 101 bp, Triticum aestivum
cggcacaacccaagcaaaccacccaatgcacgtgccttcagctcctctggyacgctcttcaagaggctctctgcttcttccagaaggccaacactcccata

SEQ ID NO: 3 - DNA, 101 bp, Triticum aestivum
tacatgatggtgttatgtatcaaccaacattacagtgcgcttgtcgactcmtggtcctttctgactgtcaatctcatgagagaattggctcgagaatttcg

SEQ ID NO: 4 - DNA, 101 bp, Triticum aestivum
tccatctttttgttgagatttactgaagaacagccgtggcaaggcgctccygtgcaaaaattcgtgctctcgtttgcctcaccagcccctgttctgtttgt

SEQ ID NO: 5 - DNA, 101 bp, Triticum aestivum
tccttcagacatcgaacacatcatcatacatgtcggcgtcccagtccgcgycgtcgatataatcctccatgtcatcaaactcggcatcctcgtcgtcgtcg

SEQ ID NO: 6 - DNA, 250 bp, Triticum aestivum
accaggtgccgcttgaaggcagatcagaagargttatgactccttcatgtacatcttggccgcgtcttgttttaggcaccggcggcagcagcagcagggagtctcttagaaccattgttgtgcaaaactggccttgccgtctcctcttccttttttcaatggagaagctgccgcaggtgcttgtggattacatttcatatgatactcactcccaccagcgcaagttgtctggaggtttttgaagtcaacg

SEQ ID NO: 7 - DNA, 101 bp, Triticum aestivum
ggcagagccggtcgacggagaggagcgccattcgacgcgtcttccgcaatrtgtttgcctgcttcggccgcggccattcggcgagctcccacgcttcgtcc

SEQ ID NO: 8 - DNA, 93 bp, Triticum aestivum
ttccggcaggtcttaaccaattccaattttcattatccaagcatagcactkaatcttgcatttratcataagcttgttgactggctaatactr

SEQ ID NO: 9 - DNA, 101 bp, Triticum aestivum
ctgaaggaaagggatccatgggtaatacaccgtgtacattctagggggtcrtgtgacagcagaatcaacttaatttttgacgagcaaccaaataccgactg

SEQ ID NO: 10 - DNA, 101 bp, Triticum aestivum; identical to SEQ ID NO: 4

SEQ ID NO: 11 - DNA, 101 bp, Triticum aestivum
tcatgtggcttgccatgttccagaacatgctgaacaacatagttaccataytgatcttgagccagcaagcaaacagactggagaatctcatccatcattat

SEQ ID NO: 12 - DNA, 101 bp, Triticum aestivum
ccaattatcaacctcctgactgtgagggaaacaaagggaatagatagattrctccagtacacatcacgaggttctggagcccattcagtcagccaaagggt

SEQ ID NO: 13 - DNA, 101 bp, Triticum aestivum
atgaagcccgggttcgatcctagcaagggtggacggccggagttttacttygaggaagggtctgatcctgagcaggtggattggataggccaaaagaacca

SEQ ID NO: 14 - DNA, 293 bp, Triticum aestivum
ttggctggtagcactgactggtcaaacctctatatatagcttatccaatggaatacatattgtccgacgtctctcttgtcaaaagtattagtggaacatttgctcgawgcctttactagacccgtccaaatgtctggtagtacacacatgaaatggaagtggtgtcgggtaaacataaactggaagtaaataaatttaacgtctctcttctccttttcgctttcgcattgtctcttttcatcaacaatgacccgcgaagataatcatcgggcacatcctttggttcctcctga

SEQ ID NO: 15 - DNA, 22463 bp, Triticum aestivum
  misc_feature (690)..(690): n is a, c, g, or t
  misc_feature (15617)..(15617): n is a, c, g, or t
  misc_feature (16309)..(16369): n is a, c, g, or t
gtagggtccgcacgcttaacgttacgatgacagttttattatgagtttataagttttgatgtaccgaagtttgttcggagtcccggatgtgatcacggacatgacgaggagtctcgaaatggtcgagacataaagattgatatattggaagcctatgtttggacatcggaaaggttccgggtgaaatcaggattttaccagaacaccggggggttaccggaaccctccaaggggttaatgggccttagtgggccatgagggagaagaggagggccggccagggcaggccacgcgccccctcccccctagtccgaataggacaaggaagggggggggggcggcgcccccctttcctctttcccctcccccctttccttctccaccaaggcaagaggggggagtcctactcccggtgggagtaggactcctccaggcgcaccccaaggggaccggctgcacctccccttccctcctttatatacgggggcaggggggcaccccataacacacaagttgatctacagatcgttccttagccgtgtgcggtgcccccctccaccatattccacctcggtcatattgtcgcggagtttaggcgaagccctgcgccggtagaacatcatcatcgtcaccacgccgtcgtgctgacggaactcatccccgaagctttgctggatcggagcccggggnagctttgctggatcggagcccggggatcgtcatcgagctgaacgtgtgctgaactcggaggtgccgtacgttcggtgcttggatcggtcggatcgtgaagacgtacgactacatcaaccgcgttgtcagaacgcttccgcttacggtctacgagggtacgtggacgaacactctcccctctcgttgctatgccatcaccatgatcttgcgtgtgcgtaggaaattttttgaaattactacgttccccaacaaggttgtgctcaggcggagcttcatgcccgccaaccgcaggagatcgccagacatggccggtgaacactgggtcccgatcgctgacgatcgaagaggggaacccgtggaggcggacgataccgtcgaagaaggcacgggccacagatgcagcagtgtaaggatgaccgagcgtgatgaagtgagcatacttggagaaattagtacaaggccttcagaaattcctccataattttgtacattttctgttaaaatttgtagatccacatgcgtaagtactggacacgcttcctcaagaagaagaatgacatagtctcctgtgatgacgctgaggccatcgccgtattcaaatccggcgtaaccgacgtgtgatactctgggggatttgatgataacccccccagttcatgtcactttgatcataaccccccctttgtgtcactgacatgtggggtctggtcccacatgtcagtgacacaaaggggggggggggttatgatcaaagtgacgtgaactgggggggttatcatcaattattccgtgatactctccagggacttcggatacttcaagcccaggaccatgccggccttgatggagatgtggcgcgtagttcgcagtatatgtgggaagacactctggatctacaaaattttaatagaaaatgtattcatttgatagccgcacacaaaaaaaaggcaaaatcatttgccattttctcttctgtaccgctcatggttcaaaagagttttcctgaattttgtaaattcatagtgtattcttgcacttcgatgtgagatcccccccccccccccccctgaaatttttgaaaactaataaatgccttttgcatatacttttttccaaataaaaggatggcttgagcttcagagccggattttttttttctcgtgcaatacttaccaaattcttgttcataaaatagtattcatagacatatatatacccaaatgtgcaacgtttcttggggatctttccatgcatgtgttacgcctgtttgttcagagaaagtatgattcagaccaaagagaaaccatttctggagtgtttctcgaagaatggttctgctaaattagtactcctacaagaatttcaggtccaagatcttcactgctaagtgagtaaatgaaaaattatgaggaaggaagaagataaaagaaaaatactgaacatgggagaaaataaattggacagtgaatataatgaaataaccaggttctgcttctacaacgcacagctaaaagaagaaaaaaagcacaccaattgttctatagtaacaaaatgcaccaaggaacaggggagaaaaccatggcaaagctcactgaaatccatcagactctgtctcaaaaaaaggtaatgagatgaatgaaccgatctactccctctgtctcataatgtaagacgttttttggcactagtgtagtgttaaaaaacatcttatattatgggacggagggagtataattttagggcacactattgttggatagaatagataataacaatgaccctgtttcattaacaaaatagtaccacatatcagtttaatatatactgcctgcttactgttcatactaccaaagccaaaaagaatagagaatttatcacctctatcggacggaatagagaagttcaaaatgcatcaaacatactatatccttattatagtcataccggcatgatatacagagtattgaataacaaaggaacatgctgacagtcgatgaaattatggacagaaccatattacctctgaacattgatatgccacagagtatgtttaattcaacgtttaaaaatgccgaggcccctgatattgatctggttaagccaagttacagggttaaactcaacatggtgctgaatcgatcaaaacaaataatttggagcccggccctaaattaatcaatgccagcatatacaaaacactaacagtcacagtcacagactgctacaacgtgatccatgtagccatacaaggcagaaggtctagaagctgcacaaataataacacaattacataagcatatgtgattcacagatcaccctattcatcaagtggctggcatataacataggagtattacccatcaacagtcaacaaaacacctgtctagtaccctgttatgattaactaacctcaaactggcttcggcagggacaagctggtcaagcacctgttgctgctcagcgttttcaaattctttctcgaaccagacaaaagagacacgctcgctgattactctgaaactttggtgtatctggtggctgagaaaacatttgcaacagctacgccgagaaattggttgactccattccctgtgaggccaagccatggatgctggcagcagaaaagggacttacacaggtgccactacatgcccggccgcctgaatctctcccgtaggtgttctactagcagacatacaacttcaaaacaattgctggtcctacagttgaattgtactctttgcgtcatcctgatggcttgttctcaactgccttcctatttacatatggaaattgcacttgttgtacaagcagataaactcatggcaaacaataattcaaccttaccttctgaggagttaagttcagatatcatgtaaaaccattcaactgtagctcattctccgcgaaactgatactttgcggggagcaatcttatctgttctctgtatttccctttccctgaaaagagagagatcagcagcgaaacagttttagcttcaagtgagtagctctttgcatcaactttagacataaggagggaggaaagtgaacctattccttggctattttggttcaccacaaatctactttccactgattcatagtgcattcttacatgtacaagtgaggtttgttcgggatgtttgattataacttacaactgtactttctgaaaaaaaaagatcaatgaatctccgaaagccggaaaaaatctgctcccagaatagaccaatttatcatttcaaagagtcccaacattcagagtacatccatatgctgctacagggtgtgctactccattacagctgcgattgcaagatctgaaatacagtcatacatattttgtgctaggtactccttcagttcagctatagtgcaaaactgaatggaattatgagatgcaaatagtactatatgattagacaattatgcccaggcaccagccaacttatggaatacaagaatgggttctctttcagaaaaatagtactggtatgatttcaggtccaagactttcactggccactgccaaggatgtttaggacgatattgaattccttctatagcttacacctacatgacccaggaaaacagtttataacattcttacgatcgcgaaaacacactagcgttctttcgtacgtactacaaaccatgttgctttacaaaaattcaaaaatcaaaacccttatttcgggaagaagaaaaagcatcatacgtataaaaaatgctaccaaaatatttactaaattctttttcaaaaaatagtattcatgcatagacatatctaccaaatgtgcaatgtttcttggggatctttccatgcatgagtcacacctgtttgttcagagacaatatgattcagacccaagacaaaccatttttggagtgtttctcgaagaatggttctactaaattagtacaagaatttcaggtccaagacctgtactactcagtgagtaaatgaaaaattacgcggaaggaacaagataaaataaaatgctgaacttctgagctctcgtaagaaaataaattagacaatgaattaatgaaataaacaggttttgttgttctataacgtacagccaaaagaaaaaaagcgcacaccaattgttctatagtaacaaaatgtaccaaggacgggcgaagctcaccgaaatccatatgagatgaatgaaccgatctataattttatggaacactattgctggataaaatagataataaaaaggaccctgtttcactaacaaaatagtaccacatatcagtttattactgcctgctttctgttcatactaccaaagccaacaagaatagaaatttatcagctttatcccaagaaacagagaagctcaaaatgcaccagccgtatatccttattatagtcataccgccgtgatatacagagtactaaataaaaaaggaacatgctgacagtcgatgaaaattacgggcagaaccatattacctctggacattgatctgcgtcagtttgtgcaacaacagagagtattgatattgtgattcctagagataacaccagcatgatctagttaagccaagttacagggttaaactcaacatggcgctgtatcgatcaaaacagaaaaattgcagaccagccctcatattaaatgccagcacatacagactacaactgcatccataaaacatgtacatggcaaagagagagccccaaaaataactagacaagcatgtatgattcagacttctgcatgcttcacaagtcaccctaatcatcaatgccagcatatacaaaacactaacagttacagattgctacaactagatccatgtagccatctacaaggcaaaaggtctagaagctgcacaaataataacacaattacataagcatatgtgattcagacttttgcatgctgcctcttcacagatcaccgtaatcatcaagaggatggcatataacatattacacatcaacagtcaataaaacacctctctagtaccctgttatgattaactaacctcaaactggttccagctgggacaagctcagctcttcaaattctttctcgaaccagacagaaggggcacactcgctgattaatctgaccatgcgtatctggccgctgaaaacaattgcatcttcaagggagccacccaaaaccgacgggaattggttgactcgattccgtgtgaggctaagccatggatggtggaagaagcaaaggcgcttagacgccagccactacatgccccgcctgacagtctcctgtagttgtttggctagcagactgtccagcttcaaaaaaaaaagtttgctgctccttctgtttgagttttgattcagtgttgttttggcagccctagttctgcctttttattggtggtgcaactgaattgtactctttgcgtcatcctgatggcttgttctaaactgacttcctatttacaaatagaaaatgcatttcttgtacaagcagacggacccatggcaagcgatgcaaattaaatttcagatatcatgtaccaactattcaactgtggctgcttcttccagaaactgatactttgtaggaagcaatttgatgtgttctctatatttccctttccttgaaaacagagagatcagcagcgaaacagttttagcttcaagtgagtagctctttgcatcaactttagacatataatttccagccttgactatctctcctttttccagtaaccttctgatgatatgatttaacaggcaagagttggcagtacagccgctcttctccatggataagaaaagattgtcagcttcttccactgaaccttcttttataagatttgtcatcattacggtgtaggtaacagcattaggaaccaagccattggctggcatagcagcaaacaaatccttagcctcttggtttctctcgaccctgtataaggcaccaataatgatattgacaattgtaatatcaaatttcacattcattgcgcttaatttccggaaaagggtgatcgcttcgctactgcagctatttctacaaagtccaccaagaattatagagtatgtatcaatgcacacacttactccagattcaaccatctcatcaaacttctcttttgcagcaacagtttgtccagccagaaataatccatccagtatgacgttataattaaaagttgtaggtttaagtcccttgtgcagcatctctttgaacagaataagcccgtcatcaatccttctatttttgcaatagccattaataagtataccatacgtaaagttacaaggttctaaaccatatgacaccatatcatcaaatactttcaatgcatctgccatcttgcggactaggcagtatccaccgatcagcaaattaaatatgataacattaggcctcataccaatgtgcactatcaagtcaaggatatcccgtgcttctgttacccttccttctgtgcataggttctgcatgattgaactgaagaacataatatcaggaggaggcatacctttcttcatcatttcagtaacatattcctttgctttcaccaaatcgccatgtgtacaaaaaccctggattaggggacgataaacagatgcgtccggtcgtactcctgtatcaatcatctgattaaactttatcacagcatcatccaacctacccttcttgcaaaatgcatgtattacggttgaatatgtgactgcatttggactcactccttgtttctgcatttcattgaagataagcatagccttatcaagcttcccagatttagcatatgcattaatcagtatgttgaatatatgacagttaggtagaatgcagtgtgttgccatggaattgaagagattgatcatgtcaactaggcatccttcggtggcatacccatgaaggcgaatagcatatgaaacgttgtcaggtttcaggcccttgatagccatggtatcaaaaattcctgcagcttctttgcttcttccatgtttgcaaagaaaggtcataaacatgttgtaagtatgcacatctgctgtaaccctccgacttgtcatctctttgaataccctaactgcctccttccagtggcctgaagaggaatatccatggatgaggctactatacgtcacattatcaggtccaacaccatcatcaatcatctgacgaaggaccacctctgccttgtccatggctctggccttgcacagcgcatcaataactgagttatatgtcaccacattaggcttaacgccctgctgcgccatttcatggaacagattgcaggccttgcttacatggccttccttaaagaagccatggataacggtgttatacgccaccacattaggagtgcagcccagctcaggcatcctgtgaagcagcacgtccagagcctcatccgcccgctttgtgtggcaaaggcccttgaggagggtgttgaagacgacttggtttgcctccaggcccgtcttgaggagacggccaaagaaggcgagcaccagatctgtgcggcaagcgcggcagcagcagtccatgaggacgccataggtgaagacatttggctgcgccacccgtcgtccgacgtctcgggacaaacggccgaagagggtgactgccagggcggggccatcgcagcaggatgcggacgcgggcgcgcgggcgagggcagccagaaatttattcaagggacgctcctggacaggattgccccgccgcagcaattcgtcaaacaggtggtgtgcgtcctccgtagtgagcgtgccagagctcgcccgctgtgccgcggcggcgaaggcggcgtggggatcccagatgcgtgagggatgagaggtggaggaggagtggcgggcgcagagtcggaggcggaggcggaggcggggtggcgacattggcgtggtggaggagaagcggggcatggccggtgtgtaggtcgcgaactcaactgggagcaggacgacggggctgtgcttttccaagttgtaccaatgtgaatgtgctaggtggcaaccttcagttatctttttttttagggtagttatcttactccctccgttcctaaataattgtctctctagagatttcaacaaatgactacatacggaacaaaatgagtgaatctacactctaaaacatgtctacatacatccgtatgttgtagtttatttgagatagctagaaagacaattatttaggaacggagggagtattatctagtactccctccgctcggaaatacttgtcagggagattgatgtatctagatgtattcttgttctagatgcatccattttcatcaaattcttcgacaagtatttccggacggagggagtatgtagtactactactactattacttactttttgcaggtaaaattaaattatggtctcatatggctatattcatatcacataatttatcagattataattttatttagaccaagaatataaatttagttgtaagccctagaaatatactaggaagccatcaaattatactagtatttttaagtattcccatagaaaaatgtatttttaagcatttagtttttttagcatctttattttttgaaagagttaaatgcactcaaggtcctaaaaaattcgtcagggtgtcactttagtcttatttcgtccaaaatgcacctttaggtcctaattctttagtaagtggtttaccctaggtcctttttctcacgagcgctcgttgacctgctcgtgtggtgcgttgacccatgccaaatcgacagaagggctgcgtaggttgctctttctttttacagaaaaccccttataaacattatcttctcattccccagtccctggctttatttcttccccaaatctgctctctctctcggcgcgcgcgtcccctaaacctatccatggccggaacttcaagctcctcggcaaggaaacaactaagatgaggagcatggcaacatcctcagcaccgccgccggcgcggcgaagcaagctccaacttcggcgggtatgttgccgctggtggtgtgtcctttttgccgtgtccgtatcaccgttatgcaaatcaaagtaaatcaaggactacaactattgattatgacaaagttatgacatattagaagagctacaggagaagatcatcgacaagattagggttcttacggtaacatggaggaggattgctcactggccgtcatagaaggggcatcttcacgggcacccacacaaattacctccagatcacctccggttgcctctgtcgctcgcctccaatgtcgccaaagtaccgtgaaagaggagagagggtgccactaagaggggggggggtctctttgcgaagcttctcgcctggcggttagaccctctatcgatgtggcatgggtcaatgcggcacgtgtgctggtcagcgagcgctcgtggaaaaggacctcgggtgaaccaattaataaagaattaggacctaaaggtgcattttggaagaaataggactaaagtgacaccccgacgaaacctttaggacctccagtgcatttaactctttttgaaacgaggtaaaagacttgccattttcactgattaagaagaagagagttgcccggttaattaaaacacgcccatcgaatagggcactccagccgacctggcactgacaagatcacacacatactgctgacgagaggacaccgtcgaggctgcaatgtcatcgtcatcgcctctccacgagcaggcaactccgatttcctcgctgacgacccatcaagacccctccgaacaaacggcacccgaggacctcgacagccaagccaaatgatcggccgcaggcgtcgaggaccgacatctccgattttgttgatgagcatcacaggagaaagttgcaagcctcacaccaagctagtccagtgcaacctgcggagagcatcgtccgccgaaaccaccctcatggagtcatcattgccgcagggcccccgccgcatgtagcttcaacttctctgtcacagtgagaaacaagcacagacgcacccaaaggggaaccgaaccgccgatatcagaaggacaagccgcgacccagcttcgcgcatcaccatcttcgtcaccgcacgagtcgcaacgccaaccactcgtatcaccggttgagcaccagccaaccatgacaccatgcacgaccagcccaaaggtagcacgggaaaggataaccggtcttcaaagcaacgccccaaagggggaaaacaccgtacggacgacatcgttgcccgacctagatgggcgaggttttcgcctgaagaaccagattcgagattgtagtaggtcgaagaactctacaacaacgccttcaacaagggaaacgacgcccataggcgccgccagcaccggccggccatagccgggcaagcttgcgcttggagcagactcaaccaacaccctcacgcagccgacacaagctggcccgcgcaatcgctggcatgcacacccctgcgcagcaaccgcgccatcgcctcacaaggcccacggcccaccatagagcacacacacccccttgctgccagaggcaaggtcaccgggatgaccgaccctgagtaagatgagagacgagctggatccgaatgaagaaccgccggatctggcgcccccttgcagcagcactacaacaaccaccaagggccggccagagcagtcgacctgcgcggagacgaatgaccaaaggaaggaaaggggggccgccaccccgcccatactcgccgagcaagagccgccggaccgaagcccaggagtttgccgacgacaccaccgcgactgccacccgctggagacgcaacttcggagaatcttcgtgccgtagccgccgcgccgcactgcgaggaggcgtgcctccctcaccatgagacccggacgctgcagagaggccccgccgccgtcgtccaccgcacaggcttagcccggcggcctcctccggcgacggcgaggtagggaggcggagggggcgcccgtgtcttcaaggaggatgtgtgggggatggggggggggggggggggggggggggggggggggggggggggggtatctttttagcatctaggtggtgaattttgtgccgtgaaatcccgcccatgttgtcccaactaaaagttggaagtctattactagtggtggccgaggttctcaacgccttcccttcttcagatgtgcctaacatgcgtaacatgaccaaatggtgttttgtgatgcgaaccatgtcttctgatgtcgttcgttgtgctccgggatcagatgcttttgggtaatcaactcatggacggggagaatggcaagatgccacacgggatgcctggaaaatgaactcggcatgatgactttctcatgacaggatggtgtcacgttgattaccccgtcgcgtcgaaagccaaatagtgctacgtcaaaatgggcagatagagatggtgaatcaagccattggtggtgtcagtcctgattgaccatttggattccgcgatgatgtttaaggcattttctcactacaaaaattcccccaagatcagacatcatcatcacatctcggtatcctcttacttaagtttgcttggagctccatcttgggttgtggtgacccaagtattaaattttgttgttgggtataacactggatctacaaaattttcatagaaaatgcatgcatctgatagctgcacaaattattattttttgcaaacatacagtgatccataatatctgcaaacagaccctaatgtctgctattctagatcacgccattttcttttctgtaccgctcatggtccaaacgagtttcttctgaattttgtgaacttagtagatttcttcttacacttagggtgcgtttggaagccgaagtatttttgtggttttctggaatactgtggtttttgaaaaaaactttggtatttaatactttgagtcgtttggataaaaaaaatactgcagttcaacaaaccatgatatctctaaaactgtggtatttttgttgtatataaaaaagaggccctgacctcttttttttaaaaccgagaaagcgctggctgctggtctctcttgtgtccaacttctggccatcaacgactgtgatgcataaatcgataggtagcccatcgatatgtccggctggaggcggatgtactcgtacacgagctgcaaacgtcgaccttcagtgcatgtgttaactacctcggtctttgattgattacaagagataactctactgtagatcttagcatctaggagaacatgctcatgcaaggctgaatgcatacgatggctattagtacaagctgatccctgagtgtagctgaatatgcatgcatgtaacagtcgatgcaaaccaaagaaaactgagaaaaactgccacttgccaaacacctcgcagttttatcaaaactgagaaaaactatggtttttagaaactgaagtatttattgaccatgtattgaaatacttaggttttggaataccatggttttgaaaaaacgttgttgagatgtgacatccccccccccctcctccaaagtttttgaaaaaaaaactaaaaataatgatatttaatatattttcctaaaataaaaggatgaattgagctctggagccaaaaaaatcttccgaaatatttaccaaattcttgttcacaaagtagtattcatggacatatacagaaccaaaatgtgtaatgtttctgggggatctttccatgtatgttattgttgcaagcattcaacactaattgtaattcactgtattagtcgcgccagtttattcagagcagacaaacatgtgcatggagctgcggaaaccattttttggagtgtttctcaaagaacagtctgcttctgaaattagtacaaaaaattcaggtccaagaccttcacttctcagcgagtaatgaactattatgaggaaaaggaaaaggctgaacttgagctctcctaacatataaaaataaaaaggcaatcaatataacaagataatgggattctgcggttcagcataaagaaagactgttctgcatcagactccgccccctggaaaaagaggtaagatgaatggactgatctatgaattaggacacactttttgttggagaaatacacactactatagctggatccatacaacctgttaatatgcagtggcataactgaatggacagtgcctctgagttcttcaaaattgttccaacttccttagggagctggatacacgaagaccatattcatagtctgtctattatgaatttaacatttctttttctttttcgaggaggtgattatcagaaccaagagcaaaataaccccaatcctaaatggtatgtattatcgcttgcctaaaagatgaaaactagtgacgaaacctaaatcaagatgagcatggtataaatggtaaaacgggagcaattccaagcatgtgcccttggatggtgttgcagatgtagtagaagaggtggagcacatgataccacggcgcagagctctgtcattgacgaggcagttcaggttcatggtggaggcacaggtgtccatgccctgcagcaaaccgatgctgttggagagcacagccaccagtatatactaccgagctacgacataaccagccccaaagaagcgtcgtgttttcaacttcctctgcaaaaaagaggatgaagtcagagtagtaaatatgcacagaaatgtaagcggttctgacagacagttgtgagataggaccctgcaaatgcaaagtagccacagtacagaaagatgtttaagcaacaagaccaaatctcctagccttcaacagtacagtacaaatttttggagtgagacatttaacacttgactctttaaaaaattgtacgaaatcaacataatgccaaatgctgcagtccaacatgcatacagaattacatcaggctcaaaggaagcacaggacctttacgttctgtctccgaggaacagaggaaaaacaaggtaaagcttcgagggccagattgctaccgctgctcaattggttgaacggatcaagcatggttacctgattttcctttgacaaaatctttatgaccttcagagcatgatgaaacatagtcaatggattcaccttttcagccttaacagctttcgtggcccatcatagtgacatcccagcttcaccttcaacctgaacacttgtgttcattaaaaaacaatttggtacacaacaactctgaattggacatagtctcgcgagcacagtagtacaattttcagatagaacccgtgacaatgatgaagtccggcatctccaagtgcccaaaaatttcatccttgatctgcaaaactattttacagagtgcaggctttgctgcccaccgagcaatacaaggcaccatgctttttcattgtcagaacgggatccaccatgttgccagattttgtccccgtattgaactgtgtccccggttggggacgtcagaacgacgctagcccccaggccagccaacattttggagccgttgaagtgcatgatccagttggagtatgcgccgtactctttagggagttcggcttcagtccattcggcgatgaagtcggccaaaacctgcgacttaatagctcgccttggcttgtaggttatgtcgaacgggaggagctcgatggcccatttggcaatccggcccgttgcgtcgcggttgtttatactatcattaaggggtacttcggatgccactgttatggagcaatcttgaaagtagtgtcgcagctttcgggatgccatgaacaccgcgtatgctatcttttgataatgcgggtaccgtgacttgcatggagttagtacagtggacacgtagtacactggtttttggagggggaacttgtgtccgtccgcttctcgttcgacgacgagcaccgcgcttacaacttgatgggttgccgcgatgtataatagcattggttcgcccgtgttgggcgcggccaggaccggatttgntacaacttgatgggttgccgcgatgtataatagcattggttcgcccgtgttgggcgcggccaggaccggatttgttgccagtatggcttttatttcttcgagtccggccgtggcagcatccgtccactcgaagtggtcggtgcgccgcaggaggcgatagaggggtaatgccttttctcctaagcgggagataaagtggcttagagccgccacgcatcctgttagtttttgtatttgtttgaggtcctttggggtattcaattgtgacagagctcggatcttggctgggtttgcttcaattcctctaccggatacgatgaagcccaagagctttccggctggtacgccgaaaacgcatttttcctggttgagcttaatgtcatatgttcggagattgtcgaacatgagccttaagtcgtctactagagtatcgacatgttttgttctgacgaccacgtcatctacgtatgcttcaactgttttgccgatctggttggccagacatgtctgaatcatgcgctgatatgttgcgccggcgtttttgagcccgaagggcatcgtgttgaagcagaatgggccgtatggggtgatgaatgccgttgcggcttggtctgactctgccatcttgatttgatggtagccagagtatgcatcgaggaaacacaatgagtcgtgtcctgcggtggcgtcgnnnnnnnnnnnnnnnnnnnnnnnnnnnnnnnnnnnnnnnnnnnnnnnnnnnnnnnnnnnnnttctttggtaccatcaccaggtttgctagccagtccggatgttttatgtctctgatgaatccggcttccagcagttttgctagctcctctcccatggcttgtctcttgggttcggaaaaacgccgtagggtctttttgacgggtttaaacccttttatgatgttcaggctgtgctcggccagcctgcgtgggattcctggcatatccgaggggtgccaggcgaaaatgtcccaattttctcgcaggaagtctctgagtgcggcgtctacatcgggtttaattgtgccccgatggaggccgtttttgtagggtccgttggatggacttggaatttgactatttcgtccgctggtttaaaagaggtggacttggatctcttgtctagtatcacatcgtccctgtccaccgtagagcgcaacgccgttaatcctcggccgctagggcctcagataatgcctccagggctagtgcggctgtcaggaccccgactcaatggcacaccgatctagcatgtaacacctcatatcattttgcggcctcacgcacggtgttcccacgggtgtcgccttaccaggcccgggaccgtttgcgccttttggctcatgtatatgatagtgttgctagcatccatatgacaaggagcccaggctgacatggctagtcgtgaacccaaagtggcactaacttacagggacaggcatacatgacccatcaacgaacgtgtcggtcatcagcgagtgaatccgggctgtagcaactgggctagcaggactccggtaaaccggactgtagcaggctaacaggactccggtagacaccgcgtgacatttccccgaagggacagacacaggaacgaagaaggacacatgccggccagcctaagtgttccggagcagtagcaagctatcaaggctcagtgaaagcactaggagacatttcctggtaagaaaggctaccaaggataaacaactagatagtcagatcccacacataccaagcatttcaataatatacacacaatatgctcaatatgtgcaaatacaacatggcatcacaacatgactctacaactcaagtattttattcaataggctccgaggagcaagatattacatatggaaccacgtggaactactagcgagactgaagtctctctgcaaaaaacataaattaagcaacgtgagtacaaatgtacccagcaagacttacatcagaactaactacatatgcatcagtatcaacaaaggggtggtggagtttaactgcagaaagccagatttgacacggtggctatcctgaactacgactgcaagtaactcttttgaggtggcgcacacgagtccacatattcaccatatcaatacaccactatggatccgctgccgtctccctacgagaacgccatccatagcactcacgcttatcttgcgtattttagagtatccactttcacttgtctatgaactgtacaggcaacccagaagtcctttaccgcggacacggctattcgaatagatgatattaaccctgtaggggtgtacttattcacacacgctctcaccacttaccgcagtttacacgacatgtactcggcaaccttcaagcggaagcccatcgagggtgtcggccacgacctgactaaccacacaagtctctcgtccaggtttatcgcttattcgggttccatccgcatggagatccggccggggtgtcgctcacggccccaaacgatgtgagtagggttcccaagcccaccattcgggtgccacttggtacaccgtgccactgtgcctagtctgtcccaagcccacctgtaccgggtgccacttggtatactactaacactacctacaaacaccagaaactagttgcaactcctggacagagatcaagttgattaataagctgagaggggccgagttaccggaacccaatgtgtggtagtagctgttcatggatcacaaacacagaactcagttcctgaggacggtttcaatgagacaacccaccatgtactcctacatggcctctcaccgctacctttaccaaatcttgttcacacacttagctcacacacagtaggacatgtttacacacctccgattcatccccgatgaatcagacttgactcaactctaagcaatagcaggcatgacaaacaagcatgaatgagtaggcacatcagggctcaaacaactcctactcatgctagtgggtttcatctatttactgtggcaatgacaggttatgcagaggataaatgggttcagctaccgcagcaagtaacagatgaatcgttgttgtcctaatgcagtaaaagagagtaggagcgagagagtgggattttatcggaatgaacaagggggttttgcttgcctggcacttctgaagataatatagtttcttcattggtgtcattgaactcatcgtcggtatgtcgtctattgggagggaacaaacaccgacaaacaaggaagaaacacaatcaatgcaaattacaatatgatgcatgatcatgacatggcaatatgctgtgatttgagctaatgcatctagcagtaggttaaatggagttggtttgaatccaatattcaaattcaaactccatatgtgaaggtttaaatgccatttactgatttgtcctaaacaacagctctaagttcttctaacatgcatgcaaatggtacagatggatagatggatttttcatatataatttattagatttggagctacggttgaatttctatgattttcagaagttttgaccattttctggaatttcctaaaaagaataaatccagaaaatgatttactgcgtcagcctaacgtcagaatgacattagcaggtcaacggggcacggcccgggtcaaacctgacctgtggggcccactagtcagtgactcagttatctaattgagataattagtgctaaactagccctaactaagccgtcagcagtgcggggcccatgtgtcaatggatcatctaattaactagttaattaacactaactaacctaacactaattaaaaaggggcctgggcccacacgttagtgagagagagggtcaaacccctgggcagacggggtcaaaccccgccggtcaaagcggtcaacccgccggcgaggacagatgcggcggtgggcttcggatttggtccttcgtcgaccaaatcgacggcggagataccctacgcgtagctggggagctgccgcatccagtggtgcaagcagttcggtgcggggaggccgggaacgtcggcgatcacgacaaccgcggtggccggagttcggacctcagcgagaacggcgttgcagcgcacggcaggaacaacgagtgggtgctatggactcctgacggtgtgctgagcatgttgcagtgctcgattgcggtcaaggctagctctggccgcggcggcgaggaaccacggcggcggtgagttcacggctccggtgactcgggcggctagaggtgcgtacgggcatggggagcaggggagaagaaggtggagctcacaacggggtcggtgatggtctcagcgagctcggggaggcggagacggcggcaaatcgatggcggcgatccttggtggccgaggaagggaacggcggagctagcggcatctaggggcttccggcgcctttcgtctgggtgaggatgaagaggggggcgaggcggagcttcctggggcgtcggcgaggcggggaggtggctgtggccgtggcgaacggcgtcggtggtgacggtggcgctcgagcacgagttgcagagcgagagggagagcagcagggaaggggatgagcatgggagggagtcgagaggggcctgagggggtgcgtggcactgcggaagacatccaggggggaggaggcagccaggcagggaggaactggcctcctcggccgcgcgcgtgcgagcacgcagctgctcctactggcaggaggaagacgacaggagggagagcagtggtggtttgggccagatggctgggccgccagctgggccggccaggtgggctgcacgggtgaggccaggtactaactctctctctcttttatttcagttttctattttgttattttgttctgggctttattaaaaatgccagggcatttccaaaaatcatgaaactaatcatggatactgtttagaataaaagcaacagtaaacattttagtttatgattatttgagcatttaaaatatttaatagcatttaaatgcccaaatgcaaatagagtatgatttaacccagagcccaaatatgtcatggaaaaatgtgcaccacctctggttattgcttctagcattttccagaaaagatgaacatttttgaaagccatttggattcacagaaaatatttttaggttgaacctatttgaattccatttggtactagggtttggacatccccatttcaagtttctttcaaagtttaaacatgatgcacacatgaagggctagcctactgcagaccaggaccaggtatgtgacaactcacccccactaagcaaaaatctcgtcccgagattcaagcatagggtaagatgaagggggaacgcaaactaacacaatcttcacaatccaggttgcacttcataggggcgttgattcgatcaccatctttgactcgatgtcttcctctgagaactccaactaacaagacaagaagaggaaaggaaaactctagaagaattgatcttctcgaagaccgaacaactcaggatcaactcatgggatgagacatagcagcatcccccgagctgagacacgaggcatacatctagagggatggagtggaacagatgacgagggttcactaggtagacaataattccacacttaagaaggtggtaaacgattgtcaacgtagcgaggagttgagttgccatgataccataacggggcaccttagggaaggtgatttgtagaaatatccccttaagtggcaaaaagaattacctttgatttagagatcattgaaactctttataccagcctaaggcaattcttgagcgatcgtttggagggggtcggtagaatggcatgctttgattagaatggatgatgtggattaccttgttgaaaacaacacaagggatgactttagtaactgaggagaagctcaacagtagagagtgagtccactgtttgagaagttatagcataaccgaggaagctgagagcaaacccagttagtgccgatgataacacctagcgcttgcgcatgctctcaagaacttgagcatttccatattcatcaaggttttaccaacatctgtgtcaaggatcctggcaacacaacatactaccatgatggatagtgatggatgatgtatatgcataggaagataacatcttctcagatttcaccttagcgaggccaaggaaacaaaatctggatgatcgaccgagagacatttagcactccgcttctaatgttctccttgatgtgctagcgtaatccatagataattatggtttgatatctagaacatcaagtaaaaggtcggacttcgggaacacaaaaatccataaggaacaactagggagtaatcctacgaaatccttatggggaggtggccaacttcctcaaacaagatactacaataataggtcttccggctgggtgtgttggccatgacatccactttaccggttatcgagggaccaaaattatagttcttgggaaaacgttccaaccatcatatctgcctgagattcagatctggttggtgtcagaatattccagactcatcaagtctagaaggaaaaatgaaagcttgcaacacaaatcgatgagatggtgttgcgaaattctcggggaatgatctacagtagtaagctccaaaacatgagctggttctgctacacacatgtgaacatgttatcccagacaagcatgaccacatggtagtcttacaacaaaacactaccgagttctggttgggaaccatcatcgaggatatcggagtcttgtgcatgatctagaattaacacaaccaattccttttccttgagcaaatcaatcagtggcttggggtgctagggaatacatatgggatgaaggttgcaagtctccaaaccac

SEQ ID NO: 16 - DNA, 2346 bp, Triticum aestivum
  CDS (1)..(2346)
atgtcgccaccccgcctccgcctccgcctccgactctgcgcccgccactcctcctccacctctcatccctcacgcatctgggatccccacgccgccttcgccgccgcggcacagcgggcgagctctggcacgctcactacggaggacgcacaccacctgtttgacgaattgctgcggcggggcaatcctgtccaggagcgtcccttgaataaatttctggctgccctcgcccgcgcgcccgcgtccgcatcctgctgcgatggccccgccctggcagtcaccctcttcggccgtttgtcccgagacgtcggacgacgggtggcgcagccaaatgtcttcacctatggcgtcctcatggactgctgctgccgcgcttgccgcacagatctggtgctcgccttctttggccgtctcctcaagacgggcctggaggcaaaccaagtcgtcttcaacaccctcctcaagggcctttgccacacaaagcgggcggatgaggctctggacgtgctgcttcacaggatgcctgagctgggctgcactcctaatgtggtggcgtataacaccgttatccatggcttctttaaggaaggccatgtaagcaaggcctgcaatctgttccatgaaatggcgcagcagggcgttaagcctaatgtggtgacatataactcagttattgatgcgctgtgcaaggccagagccatggacaaggcagaggtggtccttcgtcagatgattgatgatggtgttggacctgataatgtgacgtatagtagcctcatccatggatattcctcttcaggccactggaaggaggcagttagggtattcaaagagatgacaagtcggagggttacagcagatgtgcatacttacaacatgtttatgacctttctttgcaaacatggaagaagcaaagaagctgcaggaatttttgataccatggctatcaagggcctgaaacctgacaacgtttcatatgctattcgccttcatgggtatgccaccgaaggatgcctagttgacatgatcaatctcttcaattccatggcaacacactgcattctacctaactgtcatatattcaacatactgattaatgcatatgctaaatctgggaagcttgataaggctatgcttatcttcaatgaaatgcagaaacaaggagtgagtccaaatgcagtcacatattcaaccgtaatacatgcattttgcaagaagggtaggttggatgatgctgtgataaagtttaatcagatgattgatacaggagtacgaccggacgcatctgtttatcgtcccctaatccagggtttttgtacacatggcgatttggtgaaagcaaaggaatatgttactgaaatgatgaagaaaggtatgcctcctcctgatattatgttcttcagttcaatcatgcagaacctatgcacagaaggaagggtaacagaagcacgggatatccttgacttgatagtgcacattggtatgaggcctaatgttatcatatttaatttgctgatcggtggatactgcctagtccgcaagatggcagatgcattgaaagtatttgatgatatggtgtcatatggtttagaaccttgtaactttacgtatggtatacttattaatggctattgcaaaaatagaaggattgatgacgggcttattctgttcaaagagatgctgcacaagggacttaaacctacaacttttaattataacgtcatactggatggattatttctggctggacaaactgttgctgcaaaagagaagtttgatgagatggttgaatctggagtaagtgtgtgcattgatacatactctataattcttggtggactttgtagaaatagctgcagtagcgaagcgatcacccttttccggaaattaagcgcaatgaatgtgaaatttgatattacaattgtcaatatcattattggtgccttatacagggtcgagagaaaccaagaggctaaggatttgtttgctgctatgccagccaatggcttggttcctaatgctgttacctacaccgtaatgatgacaaatcttataaaagaaggttcagtggaagaagctgacaatcttttcttatccatggagaagagcggctgtactgccaactcttgcctgttaaatcatatcatcagaaggttactggaaaaaggagagatagtcaaggctggaaattatatgtctaaagttgatgcaaagagctactcacttgaagctaaaactgtttcgctgctgatctctctgttttcaaggaaagggaaatatagagaacacatcaaattgcttcctacaaagtatcagtttctggaagaagcagccacagttgaatag

SEQ ID NO: 17 - protein, 781 aa, Triticum aestivum
MSPPRLRLRLRLCARHSSSTSHPSRIWDPHAAFAAAAQRASSGTLTTEDAHHLFDELLRRGNPVQERPLNKFLAALARAPASASCCDGPALAVTLFGRLSRDVGRRVAQPNVFTYGVLMDCCCRACRTDLVLAFFGRLLKTGLEANQVVFNTLLKGLCHTKRADEALDVLLHRMPELGCTPNVVAYNTVIHGFFKEGHVSKACNLFHEMAQQGVKPNVVTYNSVIDALCKARAMDKAEVVLRQMIDDGVGPDNVTYSSLIHGYSSSGHWKEAVRVFKEMTSRRVTADVHTYNMFMTFLCKHGRSKEAAGIFDTMAIKGLKPDNVSYAIRLHGYATEGCLVDMINLFNSMATHCILPNCHIFNILINAYAKSGKLDKAMLIFNEMQKQGVSPNAVTYSTVIHAFCKKGRLDDAVIKFNQMIDTGVRPDASVYRPLIQGFCTHGDLVKAKEYVTEMMKKGMPPPDIMFFSSIMQNLCTEGRVTEARDILDLIVHIGMRPNVIIFNLLIGGYCLVRKMADALKVFDDMVSYGLEPCNFTYGILINGYCKNRRIDDGLILFKEMLHKGLKPTTFNYNVILDGLFLAGQTVAAKEKFDEMVESGVSVCIDTYSIILGGLCRNSCSSEAITLFRKLSAMNVKFDITIVNIIIGALYRVERNQEAKDLFAAMPANGLVPNAVTYTVMMTNLIKEGSVEEADNLFLSMEKSGCTANSCLLNHIIRRLLEKGEIVKAGNYMSKVDAKSYSLEAKTVSLLISLFSRKGKYREHIKLLPTKYQFLEEAATVE

SEQ ID NO: 18 - DNA, 3438 bp, Triticum aestivum
caacttggaaaagcacagccccgtcgtcctgctcccagttgagttcgcgacctacacaccggccatgccccgcttctcctccaccacgccaatgtcgccaccccgcctccgcctccgcctccgactctgcgcccgccactcctcctccacctctcatccctcacgcatctgggatccccacgccgccttcgccgccgcggcacagcgggcgagctctggcacgctcactacggaggacgcacaccacctgtttgacgaattgctgcggcggggcaatcctgtccaggagcgtcccttgaataaatttctggctgccctcgcccgcgcgcccgcgtccgcatcctgctgcgatggccccgccctggcagtcaccctcttcggccgtttgtcccgagacgtcggacgacgggtggcgcagccaaatgtcttcacctatggcgtcctcatggactgctgctgccgcgcttgccgcacagatctggtgctcgccttctttggccgtctcctcaagacgggcctggaggcaaaccaagtcgtcttcaacaccctcctcaagggcctttgccacacaaagcgggcggatgaggctctggacgtgctgcttcacaggatgcctgagctgggctgcactcctaatgtggtggcgtataacaccgttatccatggcttctttaaggaaggccatgtaagcaaggcctgcaatctgttccatgaaatggcgcagcagggcgttaagcctaatgtggtgacatataactcagttattgatgcgctgtgcaaggccagagccatggacaaggcagaggtggtccttcgtcagatgattgatgatggtgttggacctgataatgtgacgtatagtagcctcatccatggatattcctcttcaggccactggaaggaggcagttagggtattcaaagagatgacaagtcggagggttacagcagatgtgcatacttacaacatgtttatgacctttctttgcaaacatggaagaagcaaagaagctgcaggaatttttgataccatggctatcaagggcctgaaacctgacaacgtttcatatgctattcgccttcatgggtatgccaccgaaggatgcctagttgacatgatcaatctcttcaattccatggcaacacactgcattctacctaactgtcatatattcaacatactgattaatgcatatgctaaatctgggaagcttgataaggctatgcttatcttcaatgaaatgcagaaacaaggagtgagtccaaatgcagtcacatattcaaccgtaatacatgcattttgcaagaagggtaggttggatgatgctgtgataaagtttaatcagatgattgatacaggagtacgaccggacgcatctgtttatcgtcccctaatccagggtttttgtacacatggcgatttggtgaaagcaaaggaatatgttactgaaatgatgaagaaaggtatgcctcctcctgatattatgttcttcagttcaatcatgcagaacctatgcacagaaggaagggtaacagaagcacgggatatccttgacttgatagtgcacattggtatgaggcctaatgttatcatatttaatttgctgatcggtggatactgcctagtccgcaagatggcagatgcattgaaagtatttgatgatatggtgtcatatggtttagaaccttgtaactttacgtatggtatacttattaatggctattgcaaaaatagaaggattgatgacgggcttattctgttcaaagagatgctgcacaagggacttaaacctacaacttttaattataacgtcatactggatggattatttctggctggacaaactgttgctgcaaaagagaagtttgatgagatggttgaatctggagtaagtgtgtgcattgatacatactctataattcttggtggactttgtagaaatagctgcagtagcgaagcgatcacccttttccggaaattaagcgcaatgaatgtgaaatttgatattacaattgtcaatatcattattggtgccttatacagggtcgagagaaaccaagaggctaaggatttgtttgctgctatgccagccaatggcttggttcctaatgctgttacctacaccgtaatgatgacaaatcttataaaagaaggttcagtggaagaagctgacaatcttttcttatccatggagaagagcggctgtactgccaactcttgcctgttaaatcatatcatcagaaggttactggaaaaaggagagatagtcaaggctggaaattatatgtctaaagttgatgcaaagagctactcacttgaagctaaaactgtttcgctgctgatctctctgttttcaaggaaagggaaatatagagaacacatcaaattgcttcctacaaagtatcagtttctggaagaagcagccacagttgaatagttggtacatgatatctgaaatttaatttgcatcgcttgccatgggtccgtctgcttgtacaagaaatgcattttctatttgtaaataggaagtcagtttagaacaagccatcaggatgacgcaaagagtacaattcagttgcaccaccaataaaaaggcagaactagggctgccaaaacaacactgaatcaaaactcaaacagaaggagcagcaaacttttttttttgaagctggacagtctgctagccaaacaactacaggagactgtcaggcggggcatgtagtggctggcgtctaagcgcctttgcttcttccaccatccatggcttagcctcacacggaatcgagtcaaccaattcccgtcggttttgggtggctcccttgaagatgcaattgttttcagcggccagatacgcatggtcagattaatcagcgagtgtgccccttctgtctggttcgagaaagaatttgaagagctgagcttgtcccagctggaaccagtttgaggttagttaatcataacagggtactagagaggtgttttattgactgttgatgtgtaatatgttatatgccatcctcttgatgattacggtgatctgtgaagaggcagcatgcaaaagtctgaatcacatatgcttatgtaattgtgttattatttgtgcagcttctagaccttttgccttgtagatggctacatggatctagttgtagcaatctgtaactgttagtgttttgtatatgctggcattgatgattagggtgacttgtgaagcatgcagaagtctgaatcatacatgcttgtctagttatttttggggctctctctttgccatgtacatgttttatggatgcagttgtagtctgtatgtgctggcatttaatatgagggctggtctgcaatttttctgttttgatcgatacagcgccatgttgagtttaaccctgtaacttggcttaactagatcatgctggtgttatctctaggaatcacaatatc

SEQ ID NO: 19 - DNA, 2373 bp, Triticum aestivum
atgccccgcttctcctccaccacgccaatgtcgccaccccgcctccgcctccgcctccgactctgcgcccgccactcctcctccacctctcatccctcacgcatctgggatccccacgccgccttcgccgccgcggcacagcgggcgagctctggcacgctcactacggaggacgcacaccacctgtttgacgaattgctgcggcggggcaatcctgtccaggagcgtcccttgaataaatttctggctgccctcgcccgcgcgcccgcgtccgcatcctgctgcgatggccccgccctggcagtcaccctcttcggccgtttgtcccgagacgtcggacgacgggtggcgcagccaaatgtcttcacctatggcgtcctcatggactgctgctgccgcgcttgccgcacagatctggtgctcgccttctttggccgtctcctcaagacgggcctggaggcaaaccaagtcgtcttcaacaccctcctcaagggcctttgccacacaaagcgggcggatgaggctctggacgtgctgcttcacaggatgcctgagctgggctgcactcctaatgtggtggcgtataacaccgttatccatggcttctttaaggaaggccatgtaagcaaggcctgcaatctgttccatgaaatggcgcagcagggcgttaagcctaatgtggtgacatataactcagttattgatgcgctgtgcaaggccagagccatggacaaggcagaggtggtccttcgtcagatgattgatgatggtgttggacctgataatgtgacgtatagtagcctcatccatggatattcctcttcaggccactggaaggaggcagttagggtattcaaagagatgacaagtcggagggttacagcagatgtgcatacttacaacatgtttatgacctttctttgcaaacatggaagaagcaaagaagctgcaggaatttttgataccatggctatcaagggcctgaaacctgacaacgtttcatatgctattcgccttcatgggtatgccaccgaaggatgcctagttgacatgatcaatctcttcaattccatggcaacacactgcattctacctaactgtcatatattcaacatactgattaatgcatatgctaaatctgggaagcttgataaggctatgcttatcttcaatgaaatgcagaaacaaggagtgagtccaaatgcagtcacatattcaaccgtaatacatgcattttgcaagaagggtaggttggatgatgctgtgataaagtttaatcagatgattgatacaggagtacgaccggacgcatctgtttatcgtcccctaatccagggtttttgtacacatggcgatttggtgaaagcaaaggaatatgttactgaaatgatgaagaaaggtatgcctcctcctgatattatgttcttcagttcaatcatgcagaacctatgcacagaaggaagggtaacagaagcacgggatatccttgacttgatagtgcacattggtatgaggcctaatgttatcatatttaatttgctgatcggtggatactgcctagtccgcaagatggcagatgcattgaaagtatttgatgatatggtgtcatatggtttagaaccttgtaactttacgtatggtatacttattaatggctattgcaaaaatagaaggattgatgacgggcttattctgttcaaagagatgctgcacaagggacttaaacctacaacttttaattataacgtcatactggatggattatttctggctggacaaactgttgctgcaaaagagaagtttgatgagatggttgaatctggagtaagtgtgtgcattgatacatactctataattcttggtggactttgtagaaatagctgcagtagcgaagcgatcacccttttccggaaattaagcgcaatgaatgtgaaatttgatattacaattgtcaatatcattattggtgccttatacagggtcgagagaaaccaagaggctaaggatttgtttgctgctatgccagccaatggcttggttcctaatgctgttacctacaccgtaatgatgacaaatcttataaaagaaggttcagtggaagaagctgacaatcttttcttatccatggagaagagcggctgtactgccaactcttgcctgttaaatcatatcatcagaaggttactggaaaaaggagagatagtcaaggctggaaattatatgtctaaagttgatgcaaagagctactcacttgaagctaaaactgtttcgctgctgatctctctgttttcaaggaaagggaaatatagagaacacatcaaattgcttcctacaaagtatcagtttctggaagaagcagccacagttgaatag

SEQ ID NO: 20 - protein, 790 aa, Triticum aestivum
MPRFSSTTPMSPPRLRLRLRLCARHSSSTSHPSRIWDPHAAFAAAAQRASSGTLTTEDAHHLFDELLRRGNPVQERPLNKFLAALARAPASASCCDGPALAVTLFGRLSRDVGRRVAQPNVFTYGVLMDCCCRACRTDLVLAFFGRLLKTGLEANQVVFNTLLKGLCHTKRADEALDVLLHRMPELGCTPNVVAYNTVIHGFFKEGHVSKACNLFHEMAQQGVKPNVVTYNSVIDALCKARAMDKAEVVLRQMIDDGVGPDNVTYSSLIHGYSSSGHWKEAVRVFKEMTSRRVTADVHTYNMFMTFLCKHGRSKEAAGIFDTMAIKGLKPDNVSYAIRLHGYATEGCLVDMINLFNSMATHCILPNCHIFNILINAYAKSGKLDKAMLIFNEMQKQGVSPNAVTYSTVIHAFCKKGRLDDAVIKFNQMIDTGVRPDASVYRPLIQGFCTHGDLVKAKEYVTEMMKKGMPPPDIMFFSSIMQNLCTEGRVTEARDILDLIVHIGMRPNVIIFNLLIGGYCLVRKMADALKVFDDMVSYGLEPCNFTYGILINGYCKNRRIDDGLILFKEMLHKGLKPTTFNYNVILDGLFLAGQTVAAKEKFDEMVESGVSVCIDTYSIILGGLCRNSCSSEAITLFRKLSAMNVKFDITIVNIIIGALYRVERNQEAKDLFAAMPANGLVPNAVTYTVMMTNLIKEGSVEEADNLFLSMEKSGCTANSCLLNHIIRRLLEKGEIVKAGNYMSKVDAKSYSLEAKTVSLLISLFSRKGKYREHIKLLPTKYQFLEEAATVE

SEQ ID NO: 21 - DNA, 11981 bp, Triticum aestivum
gccgtacgttcggtgcttggatcggtcggatcgtgaagacgtacgactacatcaaccgcgttgtcagaacgcttccgcttacggtctacgagggtacgtggacgaacactctcccctctcgttgctatgccatcaccatgatcttgcgtgtgcgtaggaaattttttgaaattactacgttccccaacaaggttgtgctcaggcggagcttcatgcccgccaaccgcaggagatcgccagacatggccggtgaacactgggtcccgatcgctgacgatcgaagaggggaacccgtggaggcggacgataccgtcgaagaaggcacgggccacagatgcagcagtgtaaggatgaccgagcgtgatgaagtgagcatacttggagaaattagtacaaggccttcagaaattcctccataattttgtacattttctgttaaaatttgtagatccacatgcgtaagtactggacacgcttcctcaagaagaagaatgacatagtctcctgtgatgacgctgaggccatcgccgtattcaaatccggcgtaaccgacgtgtgatactctgggggatttgatgataaccccccagttcatgtcactttgatcataaccccccctttgtgtcactgacatgtggggtctggtcccacatgtcagtgacacaaaggggggggggggttatgatcaaagtgacgtgaactgggggggttatcatcaattattccgtgatactctccagggacttcggatacttcaagcccaggaccatgccggccttgatggagatgtggcgcgtagttcgcagtatatgtgggaagacactctggatctacaaaattttaatagaaaatgtattcatttgatagccgcacacaaaaaaaaggcaaaatcatttgccattttctcttctgtaccgctcatggttcaaaagagttttcctgaattttgtaaattcatagtgtattcttgcacttcgatgtgagatccccccccccccccccccccccccccccccccctgaaatttttgaaaactaataaatgccttttgcatatacttttttccaaataaaaggatggcttgagcttcagagccggattttttttttctcgtgcaatacttaccaaattcttgttcataaaatagtattcatagacatatatatacccaaatgtgcaacgtttcttggggatctttccatgcatgtgttacgcctgtttgttcagagaaagtatgattcagaccaaagagaaaccatttctggagtgtttctcgaagaatggttctgctaaattagtactcctacaagaatttcaggtccaagatcttcactgctaagtgagtaaatgaaaaattatgaggaaggaagaagataaaagaaaaatactgaacatgggagaaaataaattggacagtgaatataatgaaataaccaggttctgcttctacaacgcacagctaaaagaagaaaaaaagcacaccaattgttctatagtaacaaaatgcaccaaggaacaggggagaaaaccatggcaaagctcactgaaatccatcagactctgtctcaaaaaaaggtaatgagatgaatgaaccgatctactccctctgtctcataatgtaagacgttttttggcactagtgtagtgttaaaaaacatcttatattatgggacggagggagtataattttagggcacactattgttggatagaatagataataacaatgaccctgtttcattaacaaaatagtaccacatatcagtttaatatatactgcctgcttactgttcatactaccaaagccaaaaagaatagagaatttatcacctctatcggacggaatagagaagttcaaaatgcatcaaacatactatatccttattatagtcataccggcatgatatacagagtattgaataacaaaggaacatgctgacagtcgatgaaattatggacagaaccatattacctctgaacattgatatgccacagagtatgtttaattcaacgtttaaaaatgccgaggcccctgatattgatctggttaagccaagttacagggttaaactcaacatggtgctgaatcgatcaaaacaaataatttggagcccggccctaaattaatcaatgccagcatatacaaaacactaacagtcacagtcacagactgctacaacgtgatccatgtagccatacaaggcagaaggtctagaagctgcacaaataataacacaattacataagcatatgtgattcacagatcaccctattcatcaagtggctggcatataacataggagtattacccatcaacagtcaacaaaacacctgtctagtaccctgttatgattaactaacctcaaactggcttcggcagggacaagctggtcaagcacctgttgctgctcagcgttttcaaattctttctcgaaccagacaaaagagacacgctcgctgattactctgaaactttggtgtatctggtggctgagaaaacatttgcaacagctacgccgagaaattggttgactccattccctgtgaggccaagccatggatgctggcagcagaaaagggacttacacaggtgccactacatgcccggccgcctgaatctctcccgtaggtgttctactagcagacatacaacttcaaaacaattgctggtcctacagttgaattgtactctttgcgtcatcctgatggcttgttctcaactgccttcctatttacatatggaaattgcacttgttgtacaagcagataaactcatggcaaacaataattcaaccttaccttctgaggagttaagttcagatatcatgtaaaaccattcaactgtagctcattctccgcgaaactgatactttgcggggagcaatcttatctgttctctgtatttccctttccctgaaaagagagagatcagcagcgaaacagttttagcttcaagtgagtagctctttgcatcaactttagacataaggagggaggaaagtgaacctattccttggctattttggttcaccacaaatctactttccactgattcatagtgcattcttacatgtacaagtgaggtttgttcgggatgtttgattataacttacaactgtactttctgaaaaaaaaagatcaatgaatctccgaaagccggaaaaaatctgctcccagaatagaccaatttatcatttcaaagagtcccaacattcagagtacatccatatgctgctacagggtgtgctactccattacagctgcgattgcaagatctgaaatacagtcatacatattttgtgctaggtactccttcagttcagctatagtgcaaaactgaatggaattatgagatgcaaatagtactatatgattagacaattatgcccaggcaccagccaacttatggaatacaagaatgggttctctttcagaaaaatagtactggtatgatttcaggtccaagactttcactggccactgccaaggatgtttaggacgatattgaattccttctatagcttacacctacatgacccaggaaaacagtttataacattcttacgatcgcgaaaacacactagcgttctttcgtacgtactacaaaccatgttgctttacaaaaattcaaaaatcaaaacccttatttcgggaagaagaaaaagcatcatacgtataaaaaatgctaccaaaatatttactaaattctttttcaaaaaatagtattcatgcatagacatatctaccaaatgtgcaatgtttcttggggatctttccatgcatgagtcacacctgtttgttcagagacaatatgattcagacccaagacaaaccatttttggagtgtttctcgaagaatggttctactaaattagtacaagaatttcaggtccaagacctgtactactcagtgagtaaatgaaaaattacgcggaaggaacaagataaaataaaatgctgaacttctgagctctcgtaagaaaataaattagacaatgaattaatgaaataaacaggttttgttgttctataacgtacagccaaaagaaaaaaagcgcacaccaattgttctatagtaacaaaatgtaccaaggacgggcgaagctcaccgaaatccatatgagatgaatgaaccgatctataattttatggaacactattgctggataaaatagataataaaaaggaccctgtttcactaacaaaatagtaccacatatcagtttattactgcctgctttctgttcatactaccaaagccaacaagaatagaaatttatcagctttatcccaagaaacagagaagctcaaaatgcaccagccgtatatccttattatagtcataccgccgtgatatacagagtactaaataaaaaaggaacatgctgacagtcgatgaaaattacgggcagaaccatattacctctggacattgatctgcgtcagtttgtgcaacaacagagagtattgatattgtgattcctagagataacaccagcatgatctagttaagccaagttacagggttaaactcaacatggcgctgtatcgatcaaaacagaaaaattgcagaccagccctcatattaaatgccagcacatacagactacaactgcatccataaaacatgtacatggcaaagagagagccccaaaaataactagacaagcatgtatgattcagacttctgcatgcttcacaagtcaccctaatcatcaatgccagcatatacaaaacactaacagttacagattgctacaactagatccatgtagccatctacaaggcaaaaggtctagaagctgcacaaataataacacaattacataagcatatgtgattcagacttttgcatgctgcctcttcacagatcaccgtaatcatcaagaggatggcatataacatattacacatcaacagtcaataaaacacctctctagtaccctgttatgattaactaacctcaaactggttccagctgggacaagctcagctcttcaaattctttctcgaaccagacagaaggggcacactcgctgattaatctgaccatgcgtatctggccgctgaaaacaattgcatcttcaagggagccacccaaaaccgacgggaattggttgactcgattccgtgtgaggctaagccatggatggtggaagaagcaaaggcgcttagacgccagccactacatgccccgcctgacagtctcctgtagttgtttggctagcagactgtccagcttcaaaaaaaaaagtttgctgctccttctgtttgagttttgattcagtgttgttttggcagccctagttctgcctttttattggtggtgcaactgaattgtactctttgcgtcatcctgatggcttgttctaaactgacttcctatttacaaatagaaaatgcatttcttgtacaagcagacggacccatggcaagcgatgcaaattaaatttcagatatcatgtaccaactattcaactgtggctgcttcttccagaaactgatactttgtaggaagcaatttgatgtgttctctatatttccctttccttgaaaacagagagatcagcagcgaaacagttttagcttcaagtgagtagctctttgcatcaactttagacatataatttccagccttgactatctctcctttttccagtaaccttctgatgatatgatttaacaggcaagagttggcagtacagccgctcttctccatggataagaaaagattgtcagcttcttccactgaaccttcttttataagatttgtcatcattacggtgtaggtaacagcattaggaaccaagccattggctggcatagcagcaaacaaatccttagcctcttggtttctctcgaccctgtataaggcaccaataatgatattgacaattgtaatatcaaatttcacattcattgcgcttaatttccggaaaagggtgatcgcttcgctactgcagctatttctacaaagtccaccaagaattatagagtatgtatcaatgcacacacttactccagattcaaccatctcatcaaacttctcttttgcagcaacagtttgtccagccagaaataatccatccagtatgacgttataattaaaagttgtaggtttaagtcccttgtgcagcatctctttgaacagaataagcccgtcatcaatccttctatttttgcaatagccattaataagtataccatacgtaaagttacaaggttctaaaccatatgacaccatatcatcaaatactttcaatgcatctgccatcttgcggactaggcagtatccaccgatcagcaaattaaatatgataacattaggcctcataccaatgtgcactatcaagtcaaggatatcccgtgcttctgttacccttccttctgtgcataggttctgcatgattgaactgaagaacataatatcaggaggaggcatacctttcttcatcatttcagtaacatattcctttgctttcaccaaatcgccatgtgtacaaaaaccctggattaggggacgataaacagatgcgtccggtcgtactcctgtatcaatcatctgattaaactttatcacagcatcatccaacctacccttcttgcaaaatgcatgtattacggttgaatatgtgactgcatttggactcactccttgtttctgcatttcattgaagataagcatagccttatcaagcttcccagatttagcatatgcattaatcagtatgttgaatatatgacagttaggtagaatgcagtgtgttgccatggaattgaagagattgatcatgtcaactaggcatccttcggtggcatacccatgaaggcgaatagcatatgaaacgttgtcaggtttcaggcccttgatagccatggtatcaaaaattcctgcagcttctttgcttcttccatgtttgcaaagaaaggtcataaacatgttgtaagtatgcacatctgctgtaaccctccgacttgtcatctctttgaataccctaactgcctccttccagtggcctgaagaggaatatccatggatgaggctactatacgtcacattatcaggtccaacaccatcatcaatcatctgacgaaggaccacctctgccttgtccatggctctggccttgcacagcgcatcaataactgagttatatgtcaccacattaggcttaacgccctgctgcgccatttcatggaacagattgcaggccttgcttacatggccttccttaaagaagccatggataacggtgttatacgccaccacattaggagtgcagcccagctcaggcatcctgtgaagcagcacgtccagagcctcatccgcccgctttgtgtggcaaaggcccttgaggagggtgttgaagacgacttggtttgcctccaggcccgtcttgaggagacggccaaagaaggcgagcaccagatctgtgcggcaagcgcggcagcagcagtccatgaggacgccataggtgaagacatttggctgcgccacccgtcgtccgacgtctcgggacaaacggccgaagagggtgactgccagggcggggccatcgcagcaggatgcggacgcgggcgcgcgggcgagggcagccagaaatttattcaagggacgctcctggacaggattgccccgccgcagcaattcgtcaaacaggtggtgtgcgtcctccgtagtgagcgtgccagagctcgcccgctgtgccgcggcggcgaaggcggcgtggggatcccagatgcgtgagggatgagaggtggaggaggagtggcgggcgcagagtcggaggcggaggcggaggcggggtggcgacattggcgtggtggaggagaagcggggcatggccggtgtgtaggtcgcgaactcaactgggagcaggacgacggggctgtgcttttccaagttgtaccaatgtgaatgtgctaggtggcaaccttcagttatctttttttttagggtagttatcttactccctccgttcctaaataattgtctctctagagatttcaacaaatgactacatacggaacaaaatgagtgaatctacactctaaaacatgtctacatacatccgtatgttgtagtttatttgagatagctagaaagacaattatttaggaacggagggagtattatctagtactccctccgctcggaaatacttgtcagggagattgatgtatctagatgtattcttgttctagatgcatccattttcatcaaattcttcgacaagtatttccggacggagggagtatgtagtactactactactattacttactttttgcaggtaaaattaaattatggtctcatatggctatattcatatcacataatttatcagattataattttatttagaccaagaatataaatttagttgtaagccctagaaatatactaggaagccatcaaattatactagtatttttaagtattcccatagaaaaatgtatttttaagcatttagtttttttagcatctttattttttgaaagagttaaatgcactcaaggtcctaaaaaattcgtcagggtgtcactttagtcttatttcgtccaaaatgcacctttaggtcctaattctttagtaagtggtttaccctaggtcctttttctcacgagcgctcgttgacctgctcgtgtggtgcgttgacccatgccaaatcgacagaagggctgcgtaggttgctctttctttttacagaaaacccttataaacattatcttctcattccccagtccctggctttatttcttccccaaatctgctctctctctcggcgcgcgcgtccctaaacctatccatggccggaacttcaagctcctcggcaaggaaacaactaagatgaggagcatggcaacatcctcagcaccgccgccggcgcggcgaagcaagctccaacttcggcgggtatgttgccgctggtggtgtgtcctttttgccgtgtccgtatcaccgttatgcaaatcaaagtaaatcaaggactacaactattgattatgacaaagttatgacatattagaagagctacaggagaagatcatcgacaagattagggttcttacggtaacatggaggaggattgctcactggccgtcatagaaggggcatcttcacgggcacccacacaaattacctccagatcacctccggttgcctctgtcgctcgcctccaatgtcgccaaagtaccgtgaaagaggagagagggtgccactaagagggggggggtctctttgcgaagcttctcgcctggcggttagaccctctatcgatgtggcatgggtcaatgcggcacgtgtgctggtcagcgagcgctcgtggaaaaggacctcgggtgaaccaattaataaagaattaggacctaaaggtgcattttggaagaaataggactaaagtgacaccccgacgaaacctttaggacctccagtgcatttaactctttttgaaacgaggtaaaagacttgccattttcactgattaagaagaagagagttgcccggttaattaaaacacgcccatcgaatagggcactccagccgacctggcactgacaagatcacacacatactgctgacgagaggacaccgtcgaggctgcaatgtcatcgtcatcgcctctccacgagcaggcaactccgatttcctcgctgacgacccatcaagacccctccgaacaaacggcacccgaggacctcgacagccaagccaaatgatcggccgcaggcgtcgaggaccgacatctccgattttgttgatgagcatcacaggagaaagttgcaagcctcacaccaagctagtccagtgcaacctgcggagagcatcgtccgccgaaaccaccctcatggagtcatcattgccgcagggcccccgccgcatgtagcttcaacttctctgtcacagtgagaaacaagcacagacgcacccaaaggggaaccgaaccgccgatatcagaaggacaagccgcgacccagcttcgcgcatcaccatcttcgtcaccgcacgagtcgcaacgccaaccactcgtatcaccggttgagcaccagccaaccatgacaccatgcacgaccagcccaaaggtagcacgggaaaggataaccggtcttcaaagcaacgccccaaagggggaaaacaccgtacggacgacatcgttgcccgacctagatgggcgaggttttcgcctgaagaaccagattcgagattgtagtaggtcgaagaactctacaacaacgccttcaacaagggaaacgacgcccataggcgccgccagcaccggccggccatagccgggcaagcttgcgcttggagcagactcaaccaacaccctcacgcagccgacacaagctggcccgcgcaatcgctggcatgcacacccctgcgcagcaaccgcgccatcgcctcacaaggcccacggcccaccatagagcacacacaccccttgctgccagaggcaaggtcaccgggatgaccgaccctgagtaagatgagagacgagctggatccgaatgaagaaccgccggatctggcgcccccttgcagcagcactacaacaaccaccaagggccggccagagcagtcgacctgcgcggagacgaatgaccaaaggaaggaaaggggggccgccaccccgcccatactcgccgagcaagagccgccggaccgaagcccaggagtttgccgacgacaccaccgcgactgccacccgctggagacgcaacttcggagaatcttcgtgccgtagccgccgcgccgcactgcgaggaggcgtgcctccctcaccatgagacccggacgctgcagagaggccccgccgccgtcgtccaccgcacaggcttagcccggcggcctcctccggcgacggcgaggtagggaggcggagggggcgcccgtgtcttcaaggaggatgtgtgggggatgggggggggggggtatctttttagcatctaggtggtgaattttgtgccgtgaaatcccgcccatgttgtcccaactaaaagttggaagtctattactagtggtggccgaggttctcaacgccttcccttcttcagatgtgcctaacatgcgtaacatgaccaaatggtgttttgtgatgcgaaccatgtcttctgatgtcgttcgttgtgctccgggatcagatgcttttgggtaatcaactcatggacggggagaatggcaagatgccacacgggatgcctggaaaatgaactcggcatgatgactttctcatgacaggatggtgtcacgttgattaccccgtcgcgtcgaaagccaaatagtgctacgtcaaaatgggcagatagagatggtgaatcaagccattggtggtgtcagtcctgattgaccatttggattccgcgatgatgtttaaggcattttctcactacaaaaattcccccaagatcagacatcatcatcacatctcggtatcctcttacttaagtttgcttggagctccatcttgggttgtggtgacccaagtattaaattttgttgttgggtataacactggatctacaaaattttcatagaaaatgcatgcatctgatagctgcacaaattattattttttgcaaacatacagtgatccataatatctgcaaacagaccctaatgtctgctattctagatcacgccattttcttttctgtaccgctcatggtccaaacgagtttcttctgaattttgtgaacttagtagatttcttcttacacttagggtgcgtttggaagccgaagtatttttgtggttttctggaatactgtggtttttgaaaaaaactttggtatttaatactttgagtcgtttggataaaaaaaatactgcagttcaacaaaccatgatatctctaaaactgtggtatttttgttgtatataaaaaagaggccctgacctcttttttttaaaaccgagaaagcgctggctgctggtctctcttgtgtccaacttctggccatcaacgactgtgatgcataaa

SEQ ID NO: 22 - RNA, 18 nt, Artificial Sequence
  predicted RNA target
  misc_feature (7)..(7): n is a, c, g, or u
  misc_feature (13)..(13): n is a, c, g, or u
accuguncguaynygcau

SEQ ID NO: 23 - DNA, 895 bp, Triticum aestivum x Triticum timopheevi
tcttccagcgtttagtattcaagttcttctcttccagccccccggcccctctttgataaggaaagtttgcatttctcaaataaaaaatgacaaatatggttcgatggctcttctccactagcaggtttactgctttctatttgcacttttgtattaagtttccttatatatacgattttttattattttctatttgtctatttttctttttagtgcgttttatttcgattattcttctcccaatttgcaatcttttcggagcctccttcattattactcttcctccagagattcaggatccccaagctctagctcatttagcagggctaaacttctatctgagcctttacgagcaggatcctggatgggttacgttcattcagaacgagcttaatcacaatacccctctggaggacatacctggacggcttaagctcttcctaatggaagaaaagctgtctagtatgcgacaagatgtcattcaggaatttgtggcgctttatcaaagaatagggccttatctaccgatcgagccctacttggtcgatgaagcgcttcgttcctatctggaccatattcacgcaactgattctttcactgttctccaagcgtcttatcaagatctgcgggagaatgagggaggatctgttttctttagagatgctgtttcccacaaccgggatctccttgaggcggaaagctccgcaaggaggtgcctggaagtggaacagaggatccgatgggaagaaatccccaagagcaaggcaagtctcgaaagagctgagcacgagcatgctctcgacttgtttaagtcggaggatcttagaagggaattagaaaaaaaaagagcggggtagctcagtaattctgattcttttctcttccagcccccggg

SEQ ID NO: 24 - DNA, 24 bp, Artificial Sequence
  primer
tgatggtgttggacctgataatgt

SEQ ID NO: 25 - DNA, 22 bp, Artificial Sequence
  primer
ccagtggcctgaagaggaatat

SEQ ID NO: 26 - DNA, 21 bp, Artificial Sequence
  probe
acgtatagtagcctcatccat